European Patent Specification EP 4 100 022 B1, published March 12, 2025. Title: SIRNA, MEDICAL COMPOSITIONS, AND METHODS FOR TREATING DIABETES USING THE SAME. Applicant: Peking University. The sequence listing filed with the application follows.

SEQUENCE LISTING (27 sequences)

SEQ ID NO: 1 - RNA, 19 nt, Artificial Sequence
  Synthetic oligonucleotide
gguuacuguaguucacaaa

SEQ ID NO: 2 - RNA, 21 nt, Artificial Sequence
  Synthetic oligonucleotide
uuugugaacuacaguaaccuc

SEQ ID NO: 3 - RNA, 19 nt, Artificial Sequence
  Synthetic oligonucleotide
ggacuuugauacaauguca

SEQ ID NO: 4 - RNA, 21 nt, Artificial Sequence
  Synthetic oligonucleotide
ugacauuguaucaaaguccac

SEQ ID NO: 5 - RNA, 19 nt, Artificial Sequence
  Synthetic oligonucleotide
cauuguuucugguuauuaa

SEQ ID NO: 6 - RNA, 21 nt, Artificial Sequence
  Synthetic oligonucleotide
uuaauaaccagaaacaauggc

SEQ ID NO: 7 - RNA, 19 nt, Artificial Sequence
  Synthetic oligonucleotide
gaguaaagaugaucuugaa

SEQ ID NO: 8 - RNA, 21 nt, Artificial Sequence
  Synthetic oligonucleotide
uucaagaucaucuuuacucaa

SEQ ID NO: 9 - RNA, 19 nt, Artificial Sequence
  Synthetic oligonucleotide
gagauuugaugguaagaaa

SEQ ID NO: 10 - RNA, 21 nt, Artificial Sequence
  Synthetic oligonucleotide
uuucuuaccaucaaaucucca

SEQ ID NO: 11 - RNA, 19 nt, Artificial Sequence
  Synthetic oligonucleotide
gguuacuguaguucacaaa

SEQ ID NO: 12 - RNA, 21 nt, Artificial Sequence
  Synthetic oligonucleotide
uuugugaacuacaguaaccuc

SEQ ID NO: 13 - RNA, 19 nt, Artificial Sequence
  Synthetic oligonucleotide
ggacuuugauacaauguca

SEQ ID NO: 14 - RNA, 21 nt, Artificial Sequence
  Synthetic oligonucleotide
ugacauuguaucaaaguccac

SEQ ID NO: 15 - RNA, 19 nt, Artificial Sequence
  Synthetic oligonucleotide
cauuguuucugguuauuaa

SEQ ID NO: 16 - RNA, 21 nt, Artificial Sequence
  Synthetic oligonucleotide
uuaauaaccagaaacaauggc

SEQ ID NO: 17 - RNA, 19 nt, Artificial Sequence
  Synthetic oligonucleotide
gaguaaagaugaucuugaa

SEQ ID NO: 18 - RNA, 21 nt, Artificial Sequence
  Synthetic oligonucleotide
uucaagaucaucuuuacucaa

SEQ ID NO: 19 - RNA, 19 nt, Artificial Sequence
  Synthetic oligonucleotide
gagauuugaugguaagaaa

SEQ ID NO: 20 - RNA, 21 nt, Artificial Sequence
  Synthetic oligonucleotide
uuucuuaccaucaaaucucca

SEQ ID NO: 21 - DNA, 19 bp, Artificial Sequence
  Synthetic oligonucleotide
ggaccgagctgtcttctgg

SEQ ID NO: 22 - DNA, 21 bp, Artificial Sequence
  Synthetic oligonucleotide
cacacagaccaataggaaccc

SEQ ID NO: 23 - DNA, 19 bp, Artificial Sequence
  Synthetic oligonucleotide
gtgctggtgtggcctacag

SEQ ID NO: 24 - DNA, 19 bp, Artificial Sequence
  Synthetic oligonucleotide
attgctcggcccaatgagg

SEQ ID NO: 25 - DNA, 20 bp, Artificial Sequence
  Synthetic oligonucleotide
aacggcagcatttataaccc

SEQ ID NO: 26 - DNA, 20 bp, Artificial Sequence
  Synthetic oligonucleotide
cgatctgcagacacacactg

SEQ ID NO: 27 - DNA, 9865 bp, Mus musculus
gcaagatgtctatgaaacaggcttcagtttttctgttgatacagttcatatgctatattagacctggagcctgtgggaaagtgctggtgtggcctacagaatacagccattggataaatatgaaaataatcctggatgaacttgtccagagaggtcatgacgtcaccgttctcatatcttctgcttccatcctcattgggccgagcaatgaatcttctattaattttgaaatttattctgcacctttgagtaaagatgatcttgaatatgcttttgaaaaatgggtaggaaactggacatacgaattaaaaaaacttccattttggacatcttattcaaaactgcaaaaaatctccagtgaatattcagacatgattgaaagtttctgcaaagcagtagtttggaacaagagcctcatgaaaaaactccaaggatctaagtttgatgtcgttctagcagatgccttggttccctgtggtgagctgctatcagaactgcttaagacacctttagtatacagtctccgcttctgtcctggatacaaatgtgaaaagtacagtgggggccttccactccccccttcctatgtgcctgtggttctgtcagaactaagtgaccacatgacatttgcagaaagggtgaagaatatgttgcaggtgttgctttttgacttttggtttcaaacatttaacgagaaatcctggaatcagttttacagtgatgttctaggtaaactgtgcctttcattgttactgtgaaatcctgacttgatgtttttttgaatgagaatgtgtataggtgaatataaaggcatagaatgagattcttaattgtgagctgatagagtaaaaatagaagagaatcaaataggctcttagcaaggcaaaatactgcagagtaattatacagaacacttcagaaattactaaccatgcaaaattagacaaggaagatttctcttggtgatcatttgatctgctctacattgtctaagtataagaaactccaggtttcattgagtgctttaatatctgtaaatgagaacactacagagtcataattcattaccacaactatttgtgtagcactgaagaaaacacatttccttaagacatttactcacttagaaattaaaacatttatcaagaatgtcctgaaagcttattcacaattaaattgtaccactagaaccagaaacagtcaaggcaacttgattttcttagaatttgagttggatcatatctataaaacttaatcttaaagccttaaatcttgatagaaatgcataggtttttattattttcaaaataccttttcattaaataaaatattacctaatttattaggagaaacagtttaaatattaactgcttatacaaatacccagctataactttgagatatacaactaagttagtgatactagtctcctgtaacggacatagtacagcagggataaaagaaaattagtcattccttaccaattatcacattgcatttcaagaatcagaaaccaaaagcatagctactaaaatgtgtaaaatagactaaatattctacaaaagctgtgtttctaagcattttcaagcacctttgcaagagcaaaatttcaaatttattggtgcaacgttggaaatcaatgtaattttcacacaatatttatgttaatacaattatatcataaatcataactggaacattttaaattgcttgtctacatgacctcaactcattgcagaaatcacatgctttattccagacaaactcctttcaccatagtgtatttgtttttggttttggggtgcagggagacctacaacattaactgagatgatggggaaggcagacatatggctcgttcgaaccttctgggacttgaaatttcctcaccctttcttgcctaattttgactttgttggaggactccattgtaaaccagccaaaccactgcctaaggtaactctacattgtttcccttggtaaactgtttttccttttcatggaaacaattcttaaccactatttccagatgtttggttttatgaaacatatatcaagtggattagaactctctgacaattaagatatacattatttccttacatctctgaatcttcttactcttaagcaaagtattataccactttagaatgtggtcagtgatttaaaggtgtttaggtaactcataaaagagaatttatgctctcttcaagaacatatagtaaatgccagagacgtgttgaacagctaaagaaataaagaatcaatatcttcactaaatagaaattgtattctacttggaaacattatagtgatgaagagatgttatatacactgtgacaaacgttatacattgttatattagataaacagataagttgaagatatatccaacagagatgagatgtaatgtcctagaatccttgtgaagttacaatgacctagccaatgtacagggttagattaatgaatgaaaagaagagaggaaaaatagaaaattgaaacaaccattgaaagaatgacagacttagataagcaggacgatgacatggcaggcaggagtttttggacagcttcatgtatgcatgttccacacatggctctcttttaacctttccacttccttggagtctttctacccttaggttctgcagggatttattttttgtctttgtagtttccacatgcaaaagaaaacaacacttatctttctgtttctggcttattgattaatctcctgtcctctaaacaatagctattttcctaaattatttaataataataacatttttctatctgagtaaaacacaattatgtatatttaccaacactttgatacacattgatcacttgaagaatatctaagctaatcctatataggggaattttgaataatgatgtaataaacattattatgtagatttttcacttgcaattatttccttcagatatcaccaaagagtggcataggttaactgtatgtaacacattaatgttatttatatcaagacgcttatttatgtattttatctaattttacatttccaaatatgataaatgcataaatgttcaatttccatattatctgtaggagcatttttatagtacatacatttttgtgacattcatgataagtggattatgatggaatattgatatattttgaatttatttttttaatagctgacattattgaaagattttcagataattgtaagctatttaaatctgagggaacaactactttggatcatttgcctaagttaattgaattcttatttcttctgatgttagtttgtttttttaattagcatactctcttaaaaatttatgaatattacacaactctttagagagtctcttcattttgatagatttttttgttcttcataagcttttactataaggtactcctatttttcaattcccaaattactcccaatgctactgtggttattcaatacattactgctttttattctatgtcatggagtttctcttcttttttccctatttttatgtagtagaaacacattacttttatttagaatgtactaaagataatttcttttttttcaatgtgagaatacataattttttcaattaattaatttatttatgccccaaatgttgcctacatcgtggtccccctcttagagttcttctctatccctcatctccctctatctctccttccctacatttcttcttcttttctattccctcctttgctgctcgtccttctcatttctctcaaagaaaccacaaaaaagaaaatcaaagaaatgaacttaaaaaaataagaccaaaaatattccagcaaaacgaaaggaaagaaaaagcacacataagatttaatataaataaataaataaataaataaataaataaataaaaacatggcatttattttaggtggctaactattcctgggcttgggacctcctctggtgtatgattgatttacccagtcactactggggaaagctggttttcccctttgttatcagataccacttgcaaatagcttcttagttagaagtggaagtccatgaacattttctattctgtgcgcaggaacttcatctgccttgaacctgggcaggtcttagacatgctgctacagtctctgtgagtttatatgagcatcagtcttattatgcctggtagaccctgggatgtcattcatcccctctggatcttataaactttctccctcctactcatgatggtttgaaaatacctcctaatgaaactctaaatttcaataactctactgacaataattttttactctaattttcttatgttggtaaattgtactatagcacaaatgtactctccatgaacacatgactgctgaggcaatggatacactggtctcactaaaataattccagtaattacattatttcctctggtaatgtttgtctcagttccttagacagtgcttcccaggcagccattaatttgtgatgtcacaactgtcttcataggaaatggaagaatttgttcagagctctggagaacatggtgtggtggtgttttctctgggatcaatggttaaaaacattaaagaagaaaaggccaatgtagttgcttctgctcttgcccagattccacagaaggtaacataaagagttcactgggtggacaaatgtattgtaagtctattgaactctgaaaggattgcagtaggaaaaactgctgtgaaatataaagtaaggggttctttcctatgaatctcaaacaccacattaaaaagaaaagaatgaattgcagaagataaaatattagtctggttctgattgacattataacctgaaggatcacacttagatccagcatggttgtgcatacctgacctgttggagcttaaagagctgaggtaggtctttttcttcatatttacaaccagtttacacttcatgttgattcccaggcttttctgagtcattcagtgtgtcagtgtctcaaaaggagagaagtaaaagaaagaaaggatggaaggaaggagaaacagaagggagatgtacagttatgaggaatattatgctgaggctggaaaggtgcctcagtgatgcattaagaacacaggctgctcttccagaggaactggacttgattgctaggacttacatagtagctcataagtatccccaactcaattgccagggaatctcatgtgttcttcatgccccagacagaacagtcacagtgcatgcactgaattacatgcaggcaaaagatcatatacataaaatgaaacaaaaatatctgtaaagaaagaggaaaatatcttcttgccagtgactgatgtaggaaaacataagagaaaagataaaaaaaataggtgctgactctgcagtgaactcaggattataaaattatgaactcatcaacaggaactatgcttctagcacatcagataaacatgtttttctggatggtgaaagaggctgtaatttaagatggagtcttatgtaagcaaggacagtgtgggaagaatccagcagctcccaacgtcataaactctattgttgaattacttcctaaaagcagaagtcttttgatgtttgtaaactacatttactctattacttgatactgataccgcctattgtggagataattttttatcttacaaaacacaaagcatacagaaagtaaagactgacagttattattccagtttgtgaaacttccttgtacgttagaactcagtttgatactagacatgaaatgtattcaggacaattcaaagcatattttcaattttcctattgacaattgtttcttttttgtttttgtttttgtttttgagacaatttttcatggacagtcgttaatagactttatctgaaatgaagcatacttgctagtaagaaagaaattatttttagaaatgggaaattatatcatggtatattatgaatcaaaataaacctaattataatgaatagctgaaagaacacggaaatataggtaaaactatgtggctatgattttaaaagatgcaatattgagattatatgtaatatttacatatatcctatatataggattatatatgaaatatacataatcacataatcataaaatattactaatttaacactgttttcccagtaaggattatattaactctctaaaaatgtcatgtatacaagaatttgtcgttaattatcagatatataaaaattgtaacacagaagtggatgctcacagtcagctcttggatggatcacagggctcccaatggaggagctagagaaagtatccaaggagctaaagggatctgcaaccctatagatggaacaacattatgaactaaccagtaccccagagctcttgactctagctgcatatgtatcgaaagatgacctagtcggccatcactggaaagagaggcccattggacttgcaaactttatatgccccagtacaggggaacaccagggccaaaaagggggagtgggtgggtaggggagtggggggcggtatgggggacttttgggatagcattggaaatgtaaatgaggaaaatacctaataaaaaattaaaaaaacagaaattttaaaaaatgtataattaaatggcatgctcaagttattaggaagccatgtatagaaaatgtattatttatttcagtcttttaatatctcatactagtttagatttcccttctattaaattttatagtccatcatctggataatgttcaactgagtaatctcaattctctagaatcaaaatatgccaaagccttggatttctttaattaaataaggtagtgtctgtgtgtaacaggttctgtggagatttgatggtaagaaaccagacaccttaggatccaacactcggctctacaagtggatcccccagaatgaccttcttggtaaggcaaagttccactacagctttggggctatagtaatatacttatttgagaacagcccccttctgagccttcatattccccctgtctttaatattatgatcaataattatgtaaaacttcttctcactgcaggtcatccaaaaaccaaagcttttatagctcatggtggaaccaatggcatctatgaggcgatctaccatggcattcctattgttggtattcccttgtttggggatcaacctgataatattaaccacatagtagccaagggagcagctgttagagtggactttgatacaatgtcaactacagaccttctcactgccttgaagactgtcattaatgacccttcgtgagtctatttgttgtttgtttccttgtttgaagttgttttggttttttttaaggtttttttttcttttcttttcttttttgttttgtactatgtaaccacaagaccagccaataactgatataggtctgcttgcttctgtctcctgagtgctagaattaaaactatgtgcattcacgcttgatggtgaataactattcctttgaaaatattgctagattcacaacatcagattgatttttatcctatttgaaggagaataattttgaataactttgtgatattgcatgtctgaaatatgtgcttactttaacaataaagataccttgaatttaagtttcaataaatgagacatgataagtcttaaactattctatatacataaataatatcacaaatatatgtctattggtaacaaggacactatttcaagatagaatgtacatagtattcatgaaccatgatcttaaatgaaaagttaaacatttacccatattttctgaagttataaaacttttggtaaaactttaatttctataatgatatgtgatattgcataaccagtactgaagaaatgagagagagtattaaattattaccatacccagagaacactgttggtagtttcaaggtattccaatagacaaatgtacctaatgagaatatccagaggcaaaataacaggagaaagtgcacctggttcttccatacacagtctcctagtccaggaacacaattacattgctttccatccagtcagaagtctgctggaaattctgttcaaggaagaataataacttagcaagtgttttcaaaacatgaatctgattataaaaagaaattaggaaacagagatagaagagaagaggagaaaccaaaactagagaggagatatccagcatgagatatgaccctgtagagtttaaaagaattcagtgtccacttcttttcttaaaacttacacacacatacacacacacacacacacacacacacacacactttctcttgccaatgtttgaaatattgctcaacttcaaattaaaaataagtattctatggggaataaagcaaaaataagccaagtgtacctgaggagctggtatacaaggtaagctcattagttggaggtaaattcaggacttcattaagaccagtgtcaactacacaccaagttcaaaaaaaaacctgtactaaacaagactgtttcactgacttccctgtcactcaactgtcctccctatcacctcataaaacatagtacttgtgtgggaagtttatgccattcattttgagactcttgtgggacttttccccaaaccaataaatgttagggaagtcgacaaattagctttaattttagttgcatgcattgtcctttcagctataaagagaatgccatgagattatccagaatccaccatgaccagccaatgaagcccttggaccgagctgtcttctggatcgagtatgtcatgcgcaacaagggagccaagcaccttcgcccagctctgcatgaccttacctggttccagtaccactctctggatgtgattgggttcctattggtctgtgtggtagctgtggtattcatcattgcaaaatgttgcctcttttgttgccataagactgctaacatgggaaagaagaaaaaagagtagcttcatgaaggctgaagcagagagtcctgagagatgagcctctgccagctgcttccagcagaaacctgttgtctgtcccaggtgccttccctctgaaacaagacagggtcaggacttcattaaagatagctctcatagatgcactatatgttgaatgcacgtaaggatttatgcaagctatacactcagagctctagaagcaaaattgtgtgttcagtttagaatgttttaatgtaaatgaggaactatacccaacaacaatcactgaggttactgtagttcacaaaatttgcataggcataaagcctttgaaaaacctctctaaatattagttaattttttatgctctgtcttcatttaatgaacttatttttcttcccttccttttttcttctctttcatttttttttgtattgctcataaataatagcgttcaggtacagaacatttgaaatagactcacttttccatcaatataaggaaagccattgtttctggttattaattgggtacagcaaacttccaacaaatatttcctaaagggcctgtggtggaggctactctccttcaatcagaagcctttttcagacactaatcttcaagcatttactcttactgctcctgacataaattccagtacttgggagttcttaggcttggcaagattattgatttattttccttcttatctcttactcacaactgacctgaacactgtcattctcattctgccttttgaagtagatttaagctgccaaatgtcccattctctctcgctttgaaagtacacatccaagagaagattatctttttaagtcataccatcacctagctcatgttatatttcgtatctgaaatatcccccacagacacacaatgtactttgctgattttgtttaactcattcatacagaatttcttaccttgattcaataaaatgttaaaatctt